European Patent Specification EP 3 247 200 B1, published October 15, 2025. Title: PLANTS HAVING INCREASED TOLERANCE TO HERBICIDES. Applicant: BASF SE. The sequence listing filed with the application follows.

SEQUENCE LISTING (32 sequences)

SEQ ID NO: 1 - DNA, 1425 bp, Pseudomonas
atgcagaccctgagcattcagcatggcaccctggttacaatggatcagtatcgtcgtgttctgggtgatagctgggttcatgttcaggatggtcgtattgttgcactgggtgttcatgcagaaagcgttccgcctccggcagatcgtgttattgatgcacgtggtaaagttgttctgcctggttttatcaatgcacatacccatgttaatcagattctgctgcgtggtggtccgagtcatggtcgtcagctgtatgattggctgtttaatgttctgtatccgggtcagaaagcaatgcgtccggaagatgttgcagttgcagttcgtctgtattgtgcagaagcagttcgtagcggtattaccaccattaatgataatgcagatagcgccatttatccgggtaatattgaagcagcaatggccgtttatggtgaagttggtgttcgtgttgtttatgcccgtatgttttttgatcgtatggatggtcgcattcagggttatgttgatgcactgaaagcacgtagtccgcaggttgaactgtgtagcattatggaagaaaccgcagttgcaaaagatcgtattaccgcactgagcgatcaatatcatggtacagcaggcggtcgtattagcgtttggcctgcaccggcaattacaccggcagttaccgttgaaggtatgcgttgggcacaggcatttgcacgtgatcgtgcagttatgtggaccctgcatatggccgaaagcgatcatgatgaacgtctgcattggatgagtccggcagaatatatggaatgttatggtctgctggatgagcgcctgcaggttgcacattgtgtttattttgatcgcaaagatgttcgtctgctgcatcgtcataatgttaaagttgcaagccaggttgttagcaatgcatatctgggtagcggtgttgcaccggttccggaaatggttgaacgtggtatggcagttggtattggcaccgatgatggtaattgtaatgatagcgtgaacatgatcggcgatatgaaatttatggcccatattcatcgtgccgttcatcgtgatgcagatgttctgacaccggaaaaaattctggaaatggcaaccattgatggtgcacgtagcctgggtatggatcatgaaattggtagcattgaaaccggtaaacgtgcagatctgatcctgctggatctgcgtcatccgcagacaacaccgcatcatcatctggcagccaccattgtttttcaggcatatggtaatgaagttgacaccgttctgattgatggcaatgttgttatggaaaatcgtcgtctgagctttctgcctccggaacgtgaactggcatttctggaagaagcacagagtcgcgcaaccgcaattctgcagcgtgcaaatatggttgcaaatccggcatggcgtagcctgtga

SEQ ID NO: 2 - protein, 474 aa, Pseudomonas
MQTLSIQHGTLVTMDQYRRVLGDSWVHVQDGRIVALGVHAESVPPPADRVIDARGKVVLPGFINAHTHVNQILLRGGPSHGRQLYDWLFNVLYPGQKAMRPEDVAVAVRLYCAEAVRSGITTINDNADSAIYPGNIEAAMAVYGEVGVRVVYARMFFDRMDGRIQGYVDALKARSPQVELCSIMEETAVAKDRITALSDQYHGTAGGRISVWPAPAITPAVTVEGMRWAQAFARDRAVMWTLHMAESDHDERLHWMSPAEYMECYGLLDERLQVAHCVYFDRKDVRLLHRHNVKVASQVVSNAYLGSGVAPVPEMVERGMAVGIGTDDGNCNDSVNMIGDMKFMAHIHRAVHRDADVLTPEKILEMATIDGARSLGMDHEIGSIETGKRADLILLDLRHPQTTPHHHLAATIVFQAYGNEVDTVLIDGNVVMENRRLSFLPPERELAFLEEAQSRATAILQRANMVANPAWRSL

SEQ ID NO: 3 - protein, 473 aa, Pseudomonas
  misc_feature (16)..(16): Xaa can be any naturally occurring amino acid
  misc_feature (48)..(48): Xaa can be any naturally occurring amino acid
  misc_feature (64)..(64): Xaa can be any naturally occurring amino acid
  misc_feature (96)..(96): Xaa can be any naturally occurring amino acid
  misc_feature (128)..(128): Xaa can be any naturally occurring amino acid
  misc_feature (144)..(144): Xaa can be any naturally occurring amino acid
  misc_feature (192)..(192): Xaa can be any naturally occurring amino acid
  misc_feature (224)..(224): Xaa can be any naturally occurring amino acid
  misc_feature (336)..(336): Xaa can be any naturally occurring amino acid
  misc_feature (432)..(432): Xaa can be any naturally occurring amino acid
MQTLSIQHGTLVTMDXYRRVLGDSWVHVQDGRIVALGVHAESVPPPAXRVIDARGKVVLPGFIXAHTHVNQILLRGGPSHGRQFYDWLFNVVYPGXKAMRPEDVAVAVRLYCAEAVRSGITTINENAXSAIYPGNIEAAMAVYXEVGVRVVYARMFFDRMDGRIQGYVDALKARSPQVELCSIMEETAVAKXRITALSDQYHGTAGGRISVWPAPATTTAVTVXGMRWAQAFARDRAVMWTLHMAESDHDERIHGMSPAEYMECYGLLDERLQVAHCVYFDRKDVRLLHRHNVKVASQVVSNAYLGSGVAPVPEMVERGMAVGIGTDNGNSNDSAXMIGDMKFMAHIHRAVHRDADVLTPEKILEMATIDGARSLGMDHEIGSIETGKRADLILLDLRHLRRLSHHLAATIVFQAYGNEVDTVLIDGNVVMXNRRLSFLPPERELAFLEEAQSRATAILQRANMVANPAWRSL

SEQ ID NO: 4 - protein, 473 aa, Pseudomonas
MQTLSIQHGTLVTMDQYRRVLGDSWVHVQDGRIVALGVHAESVPPPADRVIDARGKVVLPGFINAHTHVNQILLRGGPSHGRQFYDWLFNVVYPGQKAMRPEDVAVAVRLYCAEAVRSGITTINENADSAIYPGNIEAAMAVYGEVGVRVVYARMFFDRMDGRIQGYVDALKARSPQVELCSIMEETAVAKDRITALSDQYHGTAGGRISVWPAPATTTAVTVEGMRWAQAFARDRAVMWTLHMAESDHDERIHGMSPAEYMECYGLLDERLQVAHCVYFDRKDVRLLHRHNVKVASQVVSNAYLGSGVAPVPEMVERGMAVGIGTDNGNSNDSANMIGDMKFMAHIHRAVHRDADVLTPEKILEMATIDGARSLGMDHEIGSIETGKRADLILLDLRHLRRLSHHLAATIVFQAYGNEVDTVLIDGNVVMENRRLSFLPPERELAFLEEAQSRATAILQRANMVANPAWRSL

SEQ ID NO: 5 - protein, 601 aa, Pseudomonas
ASMVTLTPLFSFSLLNCTRKASRSVMSASSWLVTCGMTTQLRCRFFDGIISALRRVTHYWRHIMQTLSIQHGTLVTMDQYRRVLGDSWVHVQDGRIVALGVHAESVPPPADRVIDARGKVVLPGFINAHTHVNQILLRGGPSHGRQFYDWLFNVVYPGQKAMRPEDVAVAVRLYCAEAVRSGITTINENADSAIYPGNIEAAMAVYGEVGVRVVYARMFFDRMDGRIQGYVDALKARSPQVELCSIMEGTAVAKDRITALSDQYHGTAGGRISVWPAPATTTAVTVEGMRWAQAFARDRAVMWTLHMAESDHDERIHGMSPAEYMECYGLLDERLQVAHCVYFDRKDVRLLHRHNVKVASQVVSNAYLGSGVAPVPEMVERGMAVGIGTDNGNSNDSVNMIGDMKFMAHIHRAVHRDADVLTPEKILEMATIDGARSLGMDHEIGSIETGKRADLILLDLRHPQTTPHHHLAATIVFQAYGNEVDTVLIDGNVVMENRRLSFLPPERELAFLEEAQSRATAILQRANMVANPAWRSLEMTPLLHPPPLEEIAAILARLGLGGGHDLDGYRIAMNAALPSFARVESLVGEGRLRAPASRRSE

SEQ ID NO: 6 - protein, 614 aa, Pseudomonas
SAATAALIMKASMVTLTPLFSFSLLNCTRKASRSVMSASSWLVTCGMTTQLRCRFFDGVISALRRVTHYWRHIMQTLSIQHGTLVTMDQYRRVLGDSWVHVQDGRIVALGVHAESVPPPADRVIDARGKVVLPGFINAHTHVNQILLRGGPSHGRQFYDWLFNVVYPGQKAMRPEDVAVAVRLYCAEAVRSGITTINENADSAIYPGNIEAAMAVYGEVGVRVVYARMFFDRMDGRIQGYVDALKARSPQVELCSIMEETAVAKDRITALSDQYHGTAGGRISVWPAPATTTAVTVEGMRWAQAFARDRAVMWTLHMAESDHDERIHGMSPADYMECYGLLDERLQVAHCVYFDRKDVRLLHRHNVKVASQVVSNAYLGSGVAPVPEMVERGMAVGIGTDNGNSNDSVNMIGDMKFMAHIHRAVHRDADVLTPEKILEMATIDGARSLGMDHEIGSIETGKRADLILLDLRHPQTTPHHHLAATIVFQAYGNEVDTVLIDGNVVMENRRLSFLPPERELAFLEEAQSRATAILQRANMVANPAWRSLEMTPLLHPPPLEEIAAILARLGLGGGHDLDGYRIAMNAALPSFARVESLVGEGRLRAPASRRSERPE

SEQ ID NO: 7 - protein, 144 aa, Pseudomonas
PHGRQFYDWLFNVLYPGQKAMRPEDVAVAVRLYCAEAVRSGITTINENADSAIYPGNIEAAMAVYGEVGVRVVYARMFFDRMDGRIQGYVDALKARSPQVELCSIMEETAVAKDRITALSDQYHGTAGGRISVWPAPATTTAVT

SEQ ID NO: 8 - protein, 144 aa, Pseudomonas
SHGRQFYDWLFNVLYPGQKAMRPEDVAVAVRLYCAEAVRSGITTINENADSAIYPGNIEAAMAVYGEVGVRVVYARMFFDRMDGRIQGYVDTLKARSPQVELCSIMEETAVAKDRITALSDQYHGTAGGRISVWPAPATTTAVT

SEQ ID NO: 9 - protein, 144 aa, Pseudomonas
PHGRQFYDWLFNVVYPGQKAMRPEDVAVAVRLYCAEAVRSGITTINENADSAIYPGNIEAAMAVYGEVGVRVVYARMFFDRMDGRIQGYVDALKARSPQVELCSIMEETAVAKDRITALSDQYHGTAGGRISVWPAPATTTAVT

SEQ ID NO: 10 - protein, 145 aa, Pseudomonas
SHGRQFYDWLFNVLYPGQKAMRPEDVAVAVRLYCAEAVRSGITTINENNADSAIYPGNIEAAMAVYGEVGVRVVYARMFFDRMDGRIQGYVDTLKARSPQVELCSIMEETAVAKDRITALSDQYHGTAGGRISVWPAPATTTAVT

SEQ ID NO: 11 - protein, 144 aa, Pseudomonas
SHGRQFYDWLFNVVYPGQKAMRPEDVAVAVRLYCAEAVRSGITTINENADSAIYPGNIEAAMAVYGEVGVRVVYARMFFDRMDGRIQGYVDALKARSPQVELCSIMEETAVAKDRITALSDQYHGTAGGRISVWPAPATTTAVT

SEQ ID NO: 12 - protein, 496 aa, Pseudomonas
MQTLSIQHGTLVTMDQYRRVLGDSWVHVQDGRIVALGVHAKSVPPPADRVIDARGKVVLPGFINAHTHVNQILLRGGPSHGRQFYDWLFNVVYPGQKAMRPEDVAVAVRLYCAEAVRSGITTINENADSAIYPGNIEAAMAVYGEVGVRVVYARMFFDRMDGRIQGYVDALKARSPQVELCSIMEETAVAKDRITALSDQYHGTAGGRISVWPAPATTTAVTVEGMRWAQAFARDRAVMWTLHMAESDHDGRIHGMSPAEYMECYGLLDERLQVAHCVYFDRKDVRLLHRHNVKVASQVVSNAYLGSGVAPVPEMVERGMAVGIGTDNGNSNDSVNMIGDMKFMAHIHRAVHRDADVLTPEKILEMATIDGARSLGMDHEIGSIETGKRADLILLDLRHPQTTPHHHLAATIVFQAYGNEVDTVLIDGNVVMENRCLSFLPPERELAFLEGAQSRATAILQRANMVANPAWRSLEMTPLLHPPPLEEIAAILARLG

SEQ ID NO: 13 - protein, 496 aa, Pseudomonas
MQTLSIQHGTLVTMDQYRRVLGDSWVHVQDGRIVALGVHAESVPPPADRVIDARGKVVLPGFINAHTHVNQILLRGGPSHGRQFYDWLFNVVYPGQKAMRPEDVAVAVRLYCAEAVRSGITTINENADSAIYPGNIEAAMAVYGEVGVRVVYARMFFDRMDGRIQGYVDALKARSPQVELCSIMEETAVAKDRITALSDQYHGTAGGRISVWPAPATTTAVTVEGMRWAQAFARDRAVMWTLHMAESDHDERIHGMSPAEYMECHGLLDERLQVAHCVYFDRKDVRLLHRHNVKVASQVVSNAYLGSGVAPVPEMVERGMAMGIGTDNGNSNDSVNMIGDMKFMAHIHRAVHRDADVLTPEKILEMATIDGARSLGMDHEIGSIETGKRADLILLDLRHPQTTPHHHLAATIVFQAYGNEVDTVLIDGNVVMENRRLSFLPPERELAFLEEAQSRATAILQRANMVANPAWRSLEMTPLLHPPPLEEIAAILARLG

SEQ ID NO: 14 - protein, 496 aa, Pseudomonas
MQTLSIQHGTLVTMDQYRRVLGDSWVHVQDGRIVALGVHAESVPPPADRVIDARGKVVLPGFINAHTHVNQILLRGGPSHGRQFYDWLFNVVYPGQKAMRPEDVAVAVRLYCAEAVRSGITTINENADSAIYPGNIEAAMAVYGEVGVRVVYARMFFDRMDGRIQGYVDALKARSPQVELCSIMEETAVAKDRITALSDQYHGTAGGRISVWPAPATTTAVTVEGMRWAQAFARDRAVMWTLHMAESDHDERIHGMSPAEYMECYGLLDERLQVAHCVYFDRKDVRLLHRHNVKVASQVVSNAYLGSGVAPVPEMVERGMAVGIGTDNGNSNDSVNMIGDMKFMAHIHRAVHRDADVLTPEKILEMATIDGARSLGMDHEIGSIETGKRADLILLDLRHPQTTPHHHLAATIVFQAYGNEVDTVLIDGNVVMENRRLSFLPPERELAFLEEAQSRATAILQRANMVANPAWRSLEMTPLLHPLPLEEIAAILARLG

SEQ ID NO: 15 - protein, 496 aa, Pseudomonas
MQTLSIQHGTLVTMDQYRRVLGDSWVHVQDGRIVALGVHAESVPPPADQVIDARGKVVLPGFINAHTHVNQILLRGGPSHGRQFHDWLFNVVYPGQKAMRPEDVAVAVRLYCAEAVRSGITTINENADSAIYPGNIEAAMAVYGEVGVRVVYARMFFDRMDGRIQGYVDALKARSPQVELCSIMEETAVAKDRITALSDQYHGTAGGRISVWPAPATTTAVTVEGMRWAQAFARDRAVMWTLHMAESDHDGRIHGMSPAEYMECYGLLDERLQVAHCVYFDRKDVRLLHRHNVKVASQVVSNAYLGSGVAPVPEMVERGMAVGIGTDNGNSNDSVNMIGDMKFMAHIHRAVHRDADVLTPEKILEMATIDGARSLGMDHEIGSIETGKRADLILLDLRHPQTTPHHHLAATIVFQAYGNEVDTVLIDGNVVMENRRLSFLPPERELAFLEEAQSRATAILQRANMVANPAWRSLEMTPLLHPPPLEEIAAILARLG

SEQ ID NO: 16 - protein, 496 aa, Pseudomonas
MQTLSIQHGTLVTMDQYRRVLGDSWVHVQDGRIVALGVHAESVPPPADRVIDARGKVVLPGFINAHTHVNQILLRGGPSHGRQFYDWLFNVVYPGQKAMRPEDVAVAVRLYCAEAVRSGITTINENADSAIYPGNIEAAMAVYGEVGVRVVYARMFFDRMDRRIQGYVDALKARSPQVELCSIMEETAVAKDRITALSDQYHGTAGGRISVWPAPATTTAVTVEGMRWAQAFARDRAVMWTLHMAESDHDERIHGMSPAEYMECYGLLDERLQVAHCVYFDRKDIRLLHRHNVKVASQAVSNAYLGSGVAPVPEMVERGMAVGIGTDNGNSNDSVNMIGDMKFMAHIHRAVHRDADVLTPEKILEMATIDGARSLGMDHEIGSIETGKRADLILLDLRHPQTTPHHHLAATIVFQAYGNEVDTVLIDGNVVMENRRLSFLPPERELAFLEEAQSRATAILQRANMVANPAWRSLEMTPLLHPPPLEEIAAILAQLG

SEQ ID NO: 17 - protein, 474 aa, Pseudomonas
MQTLSIQHGTLVTMDQYRRVLGDSWVHVQDGRIVALGVHAESVPPPADRVIDARGKVVLPGFINAHTHVNQILLRGGPSHGRQFYDWLFNVVYPGQKAMRPEDVAVAVRLYCAEAVRSGITTINENADSAIYPGNIEAAMAVYGEVGVRVVYARMFFDRMDGRIQGYVDALKARSPQVELCSIMEETAVAKDRITALSDQYHGTAGGRISVWPAPATTTAVTVEGMRWAQAFARDRAVMWTLHMAESDHDERIHGMSPAEYMECYGLLDERLQVAHCVYFDRKDVRLLHRHNVKVASQVVSNAYLGSGVAPVPEMVERGMAVGIGTDNGNSNDSVNMIGDMKFMAHIHRAVHRDADVLTPEKILEMATIDGARSLGMDHEIGSIETGKRADLILLDLRHPQTTPHHHLAATIVFQAYGNEVDTVLIDGNVVMENRRLSFLPPERELAFLEEAQSRATAILQRANMVANPAWRSL

SEQ ID NO: 18 - protein, 474 aa, Bacterial
MQTLSIQHGTLVTMDQYRRVLGDSWVHVQDGRIVALGVHAESVPPPADRVIDARGKVVLPGFINAHTHVNQILLRGGPSHGRQLYDWLFNVVYPGQRAMRPEDVAVAVRLYCAEAVRSGITTINENADSAIYPGNIEAAMAVYGEVGVRVVYARMFFDRMDGRIQGYVDALKARSPQVELCSIMEETAVAKDRITALSDQYHGTAGGRISVWPAPATTTAVTVEGMRWAQAFARDRAVMWTLHMAESDHDERLHWMSPAEYMECYGLLDERLQVAHCVYFDRKDVRLLHRHNVKVASQVVSNAYLGSGVAPVPEMVERGMAVGIGTDNGNSNDSVNMIGDMKFMAHIHRAVHRDADVLTPEKILEMATIDGARSLGMDHEIGSIETGKRADLILLDLRHPQTTPHHHLAATIVFQAYGNEVDTVLIDGNVVMENRRLSFLPPERELAFLEEAQSRATAILQRANMVANPAWRSL

SEQ ID NO: 19 - protein, 474 aa, Bacterial
MQTLSIQHGTLVTMDQYRRVLGDSWVHVQDGRIVALGVHAESVPPPADRVIDARGKVVLPGFINAHTHVNQILLRGGPSHGRQFYDWLFNVVYPGQKAMRPEDVAVAVRLYCAEAVRSGITTINENADSAIYPGNIEAAMAVYGEVGVRVVYARMFFDRMDGRIQGYVDALKARSPQVELCSIMEETAVAKDRITALSDQYHGTAGGRISVWPAPATTTAVTVEGMRWAQAFARDRAVMWTLHMAESDHDERLHWMSPAEYMECYGLLDERLQVAHCVYFDRKDVRLLHRHNVKVASQVVSNAYLGSGVAPVPEMVERGMAVGIGTDNGNSNDSVNMIGDMKFMAHIHRAVHRDADVLTPEKILEMATIDGARSLGMDHEIGSIETGKRADLILLDLRHPQTTPHHHLAATIVFQAYGNEVDTVLIDGNVVMENRRLSFLPPERELAFLEEAQSRATAILQRANMVANPAWRSL

SEQ ID NO: 20 - protein, 474 aa, Bacterial
MQTLSIQHGTLVTMDQYRRVLGDSWVHVQDGRIVALGVHAESVPPPADRVIDARGKVVLPGFINAHTHVNQILLRGGPSHGRQLYDWLFNVLYPGQKAMRPEDVAVAVRLYCAEAVRSGITTINENADSAIYPGNIEAAMAVYGEVGVRVVYARMFFDRMDGRIQGYVDALKARSPQVELCSIMEETAVAKDRITALSDQYHGTAGGRISVWPAPATTTAVTVEGMRWAQAFARDRAVMWTLHMAESDHDERLHWMSPAEYMECYGLLDERLQVAHCVYFDRKDVRLLHRHNVKVASQVVSNAYLGSGVAPVPEMVERGMAVGIGTDDGNSNDSVNMIGDMKFMAHIHRAVHRDADVLTPEKILEMATIDGARSLGMDHEIGSIETGKRADLILLDLRHPQTTPHHHLAATIVFQAYGNEVDTVLIDGNVVMENRRLSFLPPERELAFLEEAQSRATAILQRANMVANPAWRSL

SEQ ID NO: 21 - protein, 474 aa, Bacterial; identical to SEQ ID NO: 19

SEQ ID NO: 22 - protein, 474 aa, Bacterial
MQTLSIQHGTLVTMDQYRRVLGDSWVHVQDGRIVALGVHAESVPPPADRVIDARGKVVLPGFINAHTHVNQILLRGGPSHGRQLYDWLFNVVYPGQKAMRPEDVAVAVRLYCAEAVRSGITTINENADSAIYPGNIEAAMAVYGEVGVRVVYARMFFDRMDGRIQGYVDALKARSPQVELCSIMEETAVAKDRITALSDQYHGTAGGRISVWPAPATTTAVTVEGMRWAQAFARDRAVMWTLHMAESDHDERLHWMSPAEYMECYGLLDERLQVAHCVYFDRKDVRLLHRHNVKVASQVVSNAYLGSGVAPVPEMVERGMAVGIGTDNGNSNDSVNMIGDMKFMAHIHRAVHRDADVLTPEKILEMATIDGARSLGMDHEIGSIETGKRADLILLDLRHPQTTPHHHLAATIVFQAYGNEVDTVLIDGNVVMENRRLSFLPPERELAFLEEAQSRATAILQRANMVANPAWRSL

SEQ ID NO: 23 - protein, 474 aa, Bacterial
MQTLSIQHGTLVTMDQYRRVLGDSWVHVQDGRIVALGVHAESVPPPADRVIDARGKVVLPGFINAHTHVNQILLRGGPSHGRQLYDWLFNVVYPGQKAMRPEDVAVAVRLYCAEAVRSGITTINENADSAIYPGNIEAAMAVYGEVGVRVVYARMFFDRMDGRIQGYVDALKARSPQVELCPIMEETAVAKDRITALSDQYHGTAGGRISVWPAPATTTAVTVEGMRWAQAFARDRAVMWTLHMAESDHDERLHWMSPAEYMECYGLLDERLQVAHCVYFDRKDVRLLHRHNVKVASQVVSNAYLGSGVAPVPEMVERGMAVGIGTDNGNSNDSVNMIGDMKFMAHIHRAVHRDADVLTPEKILEMATIDGARSLGMDHEIGSIETGKRADLILLDLRHPQTTPHHHLAATIVFQAYGNEVDTVLIDGNVVMENRRLSFLPPERELAFLEEAQSRATAILQRANMVANPAWRSL

SEQ ID NO: 24 - protein, 474 aa, BACTERIAL; identical to SEQ ID NO: 17

SEQ ID NO: 25 - protein, 474 aa, Bacterial; identical to SEQ ID NO: 17

SEQ ID NO: 26 - protein, 481 aa, Bacterial
MTTTLYTGFHQLVTGDVAGTVLNGVDILVRDGEIIGLGPDLPRTLAPIGVGQEQGVEVVNCRGLTAYPGLINTHHHFFQAFVRNLAPLDWTQLDVLAWLRKIYPVFALVDEDCIYHSTVVSMAELIKHGCTTAFDHQYNYSRRGGPFLVDRQFDAANLLGLRFHAGRGCITLPMAEGSTIPDAMRESTDTFLADCERLVSRFHDPRPFAMQRVVVAPSSPVIAYPETFVESARLARHLGVSLHTHLGEGETPAMVARFGERSLDWCENRGFVGPDVWLAHGWEFTAADIARLAATGTGVAHCPAPVFLVGAEVTDIPAMAAAGVRVGFGVDGHASNDSSNLAECIRLAYLLQCLKASERQHPVPAPYDFLRMATQGGADCLNRPDLGALAVGRAADFFAVDLNRIEYIGANHDPRSLPAKVGFSGPVDMTVINGKVVWRNGEFPGLDEMELARAADGVFRRVIYGDPLVAALRRGTGVTPC

SEQ ID NO: 27 - protein, 403 aa, Bacterial
MSKDFDLIIRNAYLSEKDSVYDIGIVGDRIIKIEAKIEGTVKDEIDAKGNLVSPGFVDAHTHMDKSFTSTGERLPKFWSRPYTRDAAIEDGLKYYKNATHEEIKRHVIEHAHMQVLHGTLYTRTHVDVDSVAKTKAVEAVLEAKEELKDLIDIQVVAFAQSGFFVDLESESLIRKSLDMGCDLVGGVDPATRENNVEGSLDLCFKLAKEYDVDIDYHIHDIGTVGVYSINRLAQKTIENGYKGRVTTSHAWCFADAPSEWLDEAIPLYKDSGMKFVTCFSSTPPTMPVIKLLEAGINLGCASDNIRDFWVPFGNGDMVQGALIETQRLELKTNRDLGLIWKMITSEGARVLGIEKNYGIEVGKKADLVVLNSLSPQWAIIDQAKRLCVIKNGRIIVKDEVIVA

SEQ ID NO: 28 - protein, 363 aa, Bacterial
MYHIDVFRIPCHSPGDTSGLEDLIETGRVAPADIVAVMGKTEGNGCVNDYTREYATAMLAACLGRHLQLPPHEVEKRVAFVMSGGTEGVLSPHHTVFARRPAIDAHRPAGKRLTLGIAFTRDFLPEEIGRHAQITETAGAVKRAMRDAGIASIDDLHFVQVKCPLLTPAKIASARSRGCAPVTTDTYESMGYSRGASALGIALATEEVPSSMLVDESVLNDWSLSSSLASASAGIELEHNVVIAIGMSEQATSELVIAHGVMSDAIDAASVRRTIESLGIRSDDEMDRIVNVFAKAEASPDGVVRGMRHTMLSDSDINSTRHARAVTGAAIASVVGHGMVYVSGGAEHQGPAGGGPFAVIARA

SEQ ID NO: 29 - protein, 457 aa, Bacterial
MKTVEIIEGIASGRTSARDVCEEALATIGATDGLINAFTCRTVERARAEADAIDVRRARGEVLPPLAGLPYAVKNLFDIEGVTTLAGSKINRTLPPARADAVLVQRLKAAGAVLLGGLNMDEFAYGFTTENTHYGPTRNPHDTGRIAGGSSGGSGAAIAAGQVPLSLGSDTNGSIRVPASLCGVWGLKPTFGRLSRRGTYPFVHSIDHLGPLADSVEGLALAYDAMQGPDPLDPGCSASRIQPSVPVLSQGIAGLRIGVLGGWFRDNAGPAARAAVDVAALTLGASEVVMWPDAEIGRAAAFVITASEGGCLHLDDLRIRPQDFEPLSVDRFISGVLQPVAWYLRAQRFRRVYRDKVNALFRDWDILIAPATPISAPAIGTEWIEVNGTRHPCRPAMGLLTQPVSFAGCPVVAAPTWPGENDGMPIGVQLIAAPWNESLCLRAGKVLQDTGIARLKC

SEQ ID NO: 30 - protein, 605 aa, Bacterial
MNDRAPHPERSGRVTPDHLTDLASYQAAYAAGTDAADVISDLYARIKEDGENPIWISLLPLESALAMLADAQQRKDKGEALPLFGIPFGVKDNIDVAGLPTTAGCTGFARTPRQHAFVVQRLVDAGAIPIGKTNLDQFATGLNGTRTPFGIPRCVFNENYVSGGSSSGSAVAVANGTVPFSLGTDTAGSGRIPAAFNNLVGLKPTKGLFSGSGLVPAARSLDCISVLAHTVDDALAVARVAAGYDADDAFSRKAGAAALTEKSWPRRFNFGVPAAEHRQFFGDAEAEALFNKAVRKLEEMGGTCISFDYTPFRQAAELLYAGPWVAERLAAIESLADEHPEVLHPVVRDIILSAKRMSAVDTFNGIYRLADLVRAAESTWEKIDVMLLPTAPTIYTVEDMLADPVRLNSNLGFYTNFVNLMDLSAIAVPAGFRTNGLPFGVTFIGRAFEDGAIASLGKAFVEHDLAKGNAATAAPPKDTVAIAVVGAHLSDQPLNHQLTESGGKLRATTRTAPGYALYALRDATPAKPGMLRDQNAVGSIEVEIWDLPVAGFGAFVSEIPAPLGIGTITLEDGSHVKGFLCEPHAIETALDITHYGGWRAYLAAQ

SEQ ID NO: 31 - protein, 225 aa, Bacterial
MRSSKNVIKEFMRFKVRMEGTVNGHEFEIEGEGEGRPYEGHNTVKLKVTKGGPLPFAWDILSPQFQYGSKVYVKHPADIPDYKKLSFPEGFKWERVMNFEDGGVVTVTQDSSLQDGCFIYKVKFIGVNFPSDGPVMQKKTMGWEASTERLYPRDGVLKGEIHKALKLKDGGHYLVEFKSIYMAKKPVQLPGYYYVDSKLDITSHNEDYTIVEQYERTEGRHHLFL

SEQ ID NO: 32 - DNA, 3199 bp, Glycine max
aaatttaatcgcttgtcaaagaattcaaaacaacacagtctgagaattcttttgattcttccatttccctaatacaaaagtgttcaaaggactaaccgtctgagaattattttgtatccccattcacaaagtatcaaagatttaacagcctaagatctttgtcttaacacattggagggtacatcctttgtggtacaagtagagggtacatctacttgggtttgactgagaacaagagagggtacatctcttgtggattagttctagtggagggtacatccactaggttcaaagagaacaagggagggtacatcccttgtggatctttgcttgtaaaaggatttttataaggttgaaagaaatctcaaggaccgcaggtcacttggggactggatgtaggcacaggttgttgccgaaccagtataaaaactcttgtgtgtttgtcttcttcttccctactcttttactttccgctgtgcatttaatttcctcttttactttctgttaagtttctcttctactcctcattctcttaacaatttagtaaaagccttagaagagtaatttttaattagtaaaggtttaggaataattaattcaacccccccttcttaattattttgaggccactcgatccaacaggaatgacaggtctttctagcctgagcgatgaggaagaaagggagaagggttttggtaactgatcgcgtggtgggaaagcagattttggggttttaagttatgaataagacaacatcggtttcttaaacaaaaccgatgttaactttacaatgttaacatcattttttcaaaatccgatgttaactttctacagttaacatcgatttttcaataaccgatgttaagatattaaagttaacatcgggttttagaaaaaccgatttaacatcaacttgttaacattggttgtttaaaaaccgatgttaattaagtcaacttatttaccaaaatgccaccatgcttttatttacatcggttttccgaaaaaccgatgttaagcttgcgatgttaaatcaataaattgtagtaatgaatcttcatacgattcgacaaatcctagaagaatggttttacaaagaagatctcagacacaataaatgaggtcttaaatgatatcacacatgtcgtatcaaatcatgactccatttgcctatcatctaaaatatcagagcatatttgatttttaacgcatgatttgaaaaaaaaaaatcagatacaaaatatcaaacacataacacaacttttaacttttatgtttatttacatcttatcaaaataattaagagtcatgatttatctttaaaacgcaaatatcttttttactcaacaaaattataccatgacactcttcaaattagacatttgaaaaccaatttgcttagtcctcagtcctctcttctcactcccaatcaccaattgtaatctgaaaaactaaaatgtagccctcatcattgtttttctgatgataagacaaaaatatatatcattatacagagtatatatggggtattcttacatcaagcatcacagtatatgaccaaatttcagcctccccttgctaactgttataaaggtatgaaaaataatgcacatgtaaccaccattcgttctatatatgatgataacatatgctctgatttcccttttacctatgatattaaagtcctaatcttaatccaaaactcatatatgcttgcaaattaaactatctgtaattttttgttattatcaatctacaacttcgtttttacaccagaaaatagaaatgccatgtcaatgtcaaacacaactgagagtttcattttcacattttcttcttccttttggatgttcttggttcgattggaaattgaaatgaacccgttccagaaacgcctaggagaccatgtccttgtttaagcaattaaaaacataaatggagagtttttttcattgactagtcaactcaagttctgggtgatcacgttaccctaatttgttgttccccattttgtgttcccattattttatattgtcctatataaataataatagacttaaatatattttttttatttttaataaatatttgaatttatgttttttcagtaataattttttttcattaaatttttaataaaataatacttttattttttatccttgatattttattttattatatgataaattagtaaattttatgtttattttctaataaattaaagaattttgttttaatcttgactaataataaatgaaaaaaaattatcaagtaacagatacaaaatttactaaattatgagagactaaaaaagtgtcaaaaataaaaaataaaaaaattattttattaaggattcaacataaaaaattattagaaaataaaaataaaaataaaatatttattaaaaatataaaatataattaagcctaaataatatctataaagatcttggatgaaacttttcattgctgctaatgctggttaatcatttgcttattttaataagcagtgacctcactcgcagctcacacaaaattgtacattggtattattggaaagagtcgtttaagattttgttaaataggttgcaactagctcttgtatcaaaagggctacaccctcaaaattaattaaaatatcccaagaatataatagtaatttttttttgcactatggcattgttggaaatctttagataacatggtattgcgtgtagagactggcacagactgagaaggtcgaaaacaaaagaacaaggctttctttctctctctctctttcttgttcattttctctcacttgaaacatgcacacggtgctctgaaagttctaaccccaaagttgggaacacactgggacgatattatagcatatctctagaaaggtgattcttctcactctctctctccaacacactatttaaatacaactatagccctcttctttctcccatgcaacttgtcttaatttctttctcgatccccaacatcactagctagctccttttgtacacactctacaaccccacctagctacatcacttaattagttttcccatatctataaccaatttcaaattctcacccttaactagctagctatatttcataactgattattaccaactcactacatattattggctaggattcaccattagacttaaaagtagttgatttattatatatataaggg